European Patent Specification EP 3 781 197 B1, published September 10, 2025. Title: VARIANT ASPARAGINASE POLYPEPTIDES FOR MEDICAL USE. Applicant: KINDRED BIOSCIENCES, INC. The sequence listing filed with the application follows.

SEQUENCE LISTING (15 sequences)

SEQ ID NO: 1 - protein, 348 aa, Dickeya chrysanthemi
MERWFKSLFVLVLFFVFTASAADKLPNIVILATGGTIAGSAATGTQTTGYKAGALGVDTLINAVPEVKKLANVKGEQFSNMASENMTGDVVLKLSQRVNELLARDDVDGVVITHGTDTVEESAYFLHLTVKSDKPVVFVAAMRPATAISADGPMNLLEAVRVAGDKQSRGRGVMVVINDRIGSARYITKTNASTLDTFRANEEGYLGVIIGNRIYYQNRIDKLHTTRSVFDVRGLTSLPKVDILYGYQDDPEYLYDAAIQHGVKGIVYAGMGAGSVSVRGIAGMRKALEKGVVVMRSTRTGNGIVPPDEELPGLVSDSLNPAHARILLMLALTRTSDPKVIQEYFHTY

SEQ ID NO: 2 - protein, 327 aa, Erwinia chrysanthemi
ADKLPNIVILATGGTIAGSAATGTQTTGYKAGALGVDTLINAVPEVKKLANVKGEQFSNMASENMTGDVVLKLSQRVNELLARDDVDGVVITHGTDTVEESAYFLHLTVKSDKPVVFVAAMRPATAISADGPMNLLEAVRVAGDKQSRGRGVMVVINDRIGSARYITKTNASTLDTFRANEEGYLGVIIGNRIYYQNRIDKLHTTRSVFDVRGLTSLPKVDILYGYQDDPEYLYDAAIQHGVKGIVYAGMGAGSVSVRGIAGMRKALEKGVVVMRSTRTGNGIVPPDEELPGLVSDSLNPAHARILLMLALTRTSDPKVIQEYFHTY

SEQ ID NO: 3 - protein, 328 aa, Artificial Sequence
  Variant E. chrysanthemi asparaginase with no leader sequence for intracellular expression
MADKLPNIVILATGGTIAGSAATGTQTTGYKAGALGVDTLINAVPEVKKLANVKGEQFSNMASENMTGDVVLKLSQRVNELLARDDVDGVVITHGTDTVEESAYFLHLTVKSDKPVVFVAAMRPATAISADGPMNLLEAVRVAGDKQSRGRGVMVVINDRIGSARYITKTNASTLDTFRANEEGYLGVIIGNRIYYQNRIDKLHTTRSVFDVRGLTSLPKVDILYGYQDDPEYLYDAAIQHGVKGIVYAGMGAGSVSVRGIAGMRKALEKGVVVMRSTRTGNGIVPPDEELPGLVSDSLNPAHARILLMLALTRTSDPKVIQEYFHTY

SEQ ID NO: 4 - protein, 327 aa, Artificial Sequence
  Variant E. chrysanthemi asparaginase mature sequence with 3 cysteine substitutions
ADKLPNIVILATGGTIAGSAATGTQTTGYKAGALGVDTLICAVPEVKKLANVKGEQFSNMASENMTGDVVLCLSQRVNELLARDDVDGVVITHGTDTVEESAYFLHLTVKSDKPVVFVAAMRPATAISADGPMNLLEAVRVAGDKQSRGRGVMVVINDRIGSARYITKTNASTLDTFRANEEGYLGVIIGNRIYYQNRIDKLHTTRSVFDVRGLTSLPKVDILYGYQDDPEYLYDAAIQHGVKGIVYAGMGAGSVSVRGIAGMRCALEKGVVVMRSTRTGNGIVPPDEELPGLVSDSLNPAHARILLMLALTRTSDPKVIQEYFHTY

SEQ ID NO: 5 - protein, 336 aa, Artificial Sequence
  Variant E. chrysanthemi asparaginase mature sequence with 3 cysteine substitutions and N-terminal polyHis tag
MAHHHHHHHADKLPNIVILATGGTIAGSAATGTQTTGYKAGALGVDTLICAVPEVKKLANVKGEQFSNMASENMTGDVVLCLSQRVNELLARDDVDGVVITHGTDTVEESAYFLHLTVKSDKPVVFVAAMRPATAISADGPMNLLEAVRVAGDKQSRGRGVMVVINDRIGSARYITKTNASTLDTFRANEEGYLGVIIGNRIYYQNRIDKLHTTRSVFDVRGLTSLPKVDILYGYQDDPEYLYDAAIQHGVKGIVYAGMGAGSVSVRGIAGMRCALEKGVVVMRSTRTGNGIVPPDEELPGLVSDSLNPAHARILLMLALTRTSDPKVIQEYFHTY

SEQ ID NO: 6 - protein, 336 aa, Artificial Sequence
  Variant E. chrysanthemi asparaginase sequence with N-terminal polyHis tag
MAHHHHHHHADKLPNIVILATGGTIAGSAATGTQTTGYKAGALGVDTLINAVPEVKKLANVKGEQFSNMASENMTGDVVLKLSQRVNELLARDDVDGVVITHGTDTVEESAYFLHLTVKSDKPVVFVAAMRPATAISADGPMNLLEAVRVAGDKQSRGRGVMVVINDRIGSARYITKTNASTLDTFRANEEGYLGVIIGNRIYYQNRIDKLHTTRSVFDVRGLTSLPKVDILYGYQDDPEYLYDAAIQHGVKGIVYAGMGAGSVSVRGIAGMRKALEKGVVVMRSTRTGNGIVPPDEELPGLVSDSLNPAHARILLMLALTRTSDPKVIQEYFHTY

SEQ ID NO: 7 - protein, 328 aa, Artificial Sequence
  Variant E. chrysanthemi asparaginase mature sequence with 4 cysteine substitutions
MADKLPNIVILATGGTIAGSAATGTQTTGYKAGALGVDTLICAVPEVKKLANVKGEQFSNMASENMTGDVVLCLSQRVNELLARDDVDGVVITHGTDTVEESAYFLHLTVKSDKPVVFVAAMRPATAISADGPMNLLEAVRVAGDKQSRGRGVMVVINDRIGSARYITKTNASTLDTFRANEEGYLGVIIGNRIYYQNRIDKLHTTRSVFDVRGLTSLPKVDILYGYQDDPEYLYDAAIQHGVKGIVYAGMGAGSVSVRGIAGMRCALEKGVVVMRSTRTGNGIVPPDCELPGLVSDSLNPAHARILLMLALTRTSDPKVIQEYFHTY

SEQ ID NO: 8 - protein, 328 aa, Artificial Sequence
  Variant E. chrysanthemi asparaginase mature sequence with 1 lysine substitution
MADKLPNIVILATGGTIAGSAATGTQTTGYKAGALGVDTLIKAVPEVKKLANVKGEQFSNMASENMTGDVVLKLSQRVNELLARDDVDGVVITHGTDTVEESAYFLHLTVKSDKPVVFVAAMRPATAISADGPMNLLEAVRVAGDKQSRGRGVMVVINDRIGSARYITKTNASTLDTFRANEEGYLGVIIGNRIYYQNRIDKLHTTRSVFDVRGLTSLPKVDILYGYQDDPEYLYDAAIQHGVKGIVYAGMGAGSVSVRGIAGMRKALEKGVVVMRSTRTGNGIVPPDEELPGLVSDSLNPAHARILLMLALTRTSDPKVIQEYFHTY

SEQ ID NO: 9 - protein, 328 aa, Artificial Sequence
  Variant E. chrysanthemi asparaginase mature sequence with 2 lysine substitutions
MADKLPNIVILATGGTIAGSAATGTQTTGYKAGALGVDTLIKAVPEVKKLANVKGEQFSNMASENMTGDVVLKLSQRVNELLARDDVDGVVITHGTDTVEESAYFLHLTVKSDKPVVFVAAMRPATAISADGPMNLLEAVRVAGDKQSRGRGVMVVINDRIGSARYITKTNASTLDTFRANEEGYLGVIIGNRIYYQNRIDKLHTTRSVFDVRGLTSLPKVDILYGYQDDPEYLYDAAIQHGVKGIVYAGMGAGSVSVRGIAGMRKALEKGVVVMRSTRTGNGIVPPDKELPGLVSDSLNPAHARILLMLALTRTSDPKVIQEYFHTY

SEQ ID NO: 10 - protein, 348 aa, Escherichia coli
MEFFKKTALAALVMGFSGAALALPNITILATGGTIAGGGDSATKSNYTVGKVGVENLVNAVPQLKDIANVKGEQVVNIGSQDMNDNVWLTLAKKINTDCDKTDGFVITHGTDTMEETAYFLDLTVKCDKPVVMVGAMRPSTSMSADGPFNLYNAVVTAADKASANRGVLVVMNDTVLDGRDVTKTNTTDVATFKSVNYGPLGYIHNGKIDYQRTPARKHTSDTPFDVSKLNELPKVGIVYNYANASDLPAKALVDAGYDGIVSAGVGNGNLYKSVFDTLATAAKTGTAVVRSSRVPTGATTQDAEVDDAKYGFVASGTLNPQKARVLLQLALTQTKDPQQIQQIFNQY

SEQ ID NO: 11 - protein, 326 aa, Escherichia coli
LPNITILATGGTIAGGGDSATKSNYTVGKVGVENLVNAVPQLKDIANVKGEQVVNIGSQDMNDNVWLTLAKKINTDCDKTDGFVITHGTDTMEETAYFLDLTVKCDKPVVMVGAMRPSTSMSADGPFNLYNAVVTAADKASANRGVLVVMNDTVLDGRDVTKTNTTDVATFKSVNYGPLGYIHNGKIDYQRTPARKHTSDTPFDVSKLNELPKVGIVYNYANASDLPAKALVDAGYDGIVSAGVGNGNLYKSVFDTLATAAKTGTAVVRSSRVPTGATTQDAEVDDAKYGFVASGTLNPQKARVLLQLALTQTKDPQQIQQIFNQY

SEQ ID NO: 12 - protein, 326 aa, Artificial Sequence
  Variant E. coli asparaginase mature sequence with one additional cysteine pair
LPNITILCTGGTIAGGGDSATKSNYTVGKVGCENLVNAVPQLKDIANVKGEQVVNIGSQDMNDNVWLTLAKKINTDCDKTDGFVITHGTDTMEETAYFLDLTVKCDKPVVMVGAMRPSTSMSADGPFNLYNAVVTAADKASANRGVLVVMNDTVLDGRDVTKTNTTDVATFKSVNYGPLGYIHNGKIDYQRTPARKHTSDTPFDVSKLNELPKVGIVYNYANASDLPAKALVDAGYDGIVSAGVGNGNLYKSVFDTLATAAKTGTAVVRSSRVPTGATTQDAEVDDAKYGFVASGTLNPQKARVLLQLALTQTKDPQQIQQIFNQY

SEQ ID NO: 13 - protein, 321 aa, Escherichia coli
MGKAVIAIHGGAGAISRAQMSLQQELRYIEALSAIVETGQKMLEAGESALDVVTEAVRLLEECPLFNAGIGAVFTRDETHELDACVMDGNTLKAGAVAGVSHLRNPVLAARLVMEQSPHVMMIGEGAENFAFARGMERVSPEIFSTSLRYEQLLAARKEGATVLDHSGAPLDEKQKMGTVGAVALDLDGNLAAATSTGGMTNKLPGRVGDSPLVGAGCYANNASVAVSCTGTGEVFIRALAAYDIAALMDYGGLSLAEACERVVMEKLPALGGSGGLIAIDHEGNVALPFNTEGMYRAWGYAGDTPTTGIYREKGDTVATQ

SEQ ID NO: 14 - protein, 303 aa, Escherichia coli
QMSLQQELRYIEALSAIVETGQKMLEAGESALDVVTEAVRLLEECPLFNAGIGAVFTRDETHELDACVMDGNTLKAGAVAGVSHLRNPVLAARLVMEQSPHVMMIGEGAENFAFARGMERVSPEIFSTSLRYEQLLAARKEGATVLDHSGAPLDEKQKMGTVGAVALDLDGNLAAATSTGGMTNKLPGRVGDSPLVGAGCYANNASVAVSCTGTGEVFIRALAAYDIAALMDYGGLSLAEACERVVMEKLPALGGSGGLIAIDHEGNVALPFNTEGMYRAWGYAGDTPTTGIYREKGDTVATQ

SEQ ID NO: 15 - protein, 303 aa, Artificial Sequence
  Variant E. coli asparaginase mature sequence with no unpaired cysteines
QMSLQQELRYIEALSAIVETGQKMLEAGESALDVVTEAVRLLEESPLFNAGIGAVFTRDETHELDACVMDGNTLKAGAVAGVSHLRNPVLAARLVMEQSPHVMMIGEGAENFAFARGMERVSPEIFSTSLRYEQLLAARKEGATVLDHSGAPLDEKQKMGTVGAVALDLDGNLAAATSTGGMTNKLPGRVGDSPLVGAGCYANNASVAVSSTGTGEVFIRALAAYDIAALMDYGGLSLAEASERVVMEKLPALGGSGGLIAIDHEGNVALPFNTEGMYRAWGYAGDTPTTGIYREKGDTVATQ